European Patent Application EP 4 596 577 A2, published August 6, 2025. Title: Meat substitute comprising animal myoglobin. Applicant: Paleo B.V. Application EP. The sequence listing filed with the application follows.

SEQUENCE LISTING (80 sequences)

SEQ ID NO: 1 - protein, 127 aa, Mammuthus primigenius
  REGION 1..127: note = partial sequence of mammoth myoglobin
MGLSDGEWELVLKTWGKVEADIPGHGLEVFVRLFTGHPETLEKFDKFKHLKTEGEMKASEDLKKQGVTVLTALGGILKKKGHHQAEIQPLAQSHATKHKIPIKYLEFISDAIIHVLQSKHPAEFGAD

SEQ ID NO: 2 - protein, 154 aa, Mammuthus primigenius
  REGION 1..154: note = mammoth myoglobin
MGLSDGEWELVLKTWGKVEADIPGHGLEVFVRLFTGHPETLEKFDKFKHLKTEGEMKASEDLKKQGVTVLTALGGILKKKGHHQAEIQPLAQSHATKHKIPIKYLEFISDAIIHVLQSKHPAEFGADAQGAMKKALELFRNDIAAKYKELGFQG

SEQ ID NO: 3 - protein, 154 aa, Mammuthus trogontherii
  REGION 1..154: note = steppe mammoth myoglobin
MGLSDGEWELVLKTWGKVEADIPGHGLEVFVRLFTGHPETLEKFDKFKHLKTEGEMKASEDLKKQGVTVLTALGGILKKKGHHQAEIQPLAHSHATKHKIPIKYLEFISDAIIHVLQSKHPAEFGADAQGAMKKALELFRNDIAAKYKELGFQG

SEQ ID NO: 4 - protein, 154 aa, Ovis aries
  REGION 1..154: note = sheep myoglobin
MGLSDGEWQLVLNAWGKVEADVAGHGQEVLIRLFTGHPETLEKFDKFKHLKTEAEMKASEDLKKHGNTVLTALGGILKKKGHHEAEVKHLAESHANKHKIPVKYLEFISDAIIHVLHAKHPSDFGADAQGAMSKALELFRNDMAAQYKVLGFQG

SEQ ID NO: 5 - protein, 154 aa, Bos taurus
  REGION 1..154: note = cow myoglobin
MGLSDGEWQLVLNAWGKVEADVAGHGQEVLIRLFTGHPETLEKFDKFKHLKTEAEMKASEDLKKHGNTVLTALGGILKKKGHHEAEVKHLAESHANKHKIPVKYLEFISDAIIHVLHAKHPSDFGADAQAAMSKALELFRNDMAAQYKVLGFHG

SEQ ID NO: 6 - protein, 154 aa, Sus scrofa
  REGION 1..154: note = pig myoglobin
MGLSDGEWQLVLNVWGKVEADVAGHGQEVLIRLFKGHPETLEKFDKFKHLKSEDEMKASEDLKKHGNTVLTALGGILKKKGHHEAELTPLAQSHATKHKIPVKYLEFISEAIIQVLQSKHPGDFGADAQGAMSKALELFRNDMAAKYKELGFQG

SEQ ID NO: 7 - protein, 154 aa, Gallus gallus
  REGION 1..154: note = chicken myoglobin
MGLSDQEWQQVLTIWGKVEADIAGHGHEVLMRLFHDHPETLDRFDKFKGLKTPDQMKGSEDLKKHGATVLTQLGKILKQKGNHESELKPLAQTHATKHKIPVKYLEFISEVIIKVIAEKHAADFGADSQAAMKKALELFRNDMASKYKEFGFQG

SEQ ID NO: 8 - protein, 147 aa, Thunnus orientalis
  REGION 1..147: note = tuna myoglobin
MADFDAVLKCWGPVEADYTTMGGLVLTRLFKEHPETQKLFPKFAGIAQADIAGNAAISAHGATVLKKLGELLKAKGSHAAILKPLANSHATKHKIPINNFKLISEVLVKVMHEKAGLDAGQQTALRNVMGIIIADLEANYKELGFSG

SEQ ID NO: 9 - DNA, 382 bp, Mammuthus primigenius
  misc_feature 1..382: note = DNA sequence coding for partial sequence of mammoth myoglobin
  source 1..382: mol_type = other DNA
atgggactcagcgacggggaatgggagttggtgttgaaaacctgggggaaagtggaggctgacatcccgggccatgggctggaagtcttcgtcaggctcttcacaggtcatcccgagaccctggagaagttcgacaagtttaagcacctgaagacagagggcgagatgaaggcctctgaggacctgaagaagcaaggtgttactgtgctcactgccctggggggcatcctcaagaagaaagggcatcaccaggcggagattcagcccctggcccagtctcatgccaccaagcacaagatccccatcaagtatctggagttcatctcggacgccatcatccacgttctgcaaagcaagcatcctgcggaatttggcgctgatg

SEQ ID NO: 10 - DNA, 465 bp, Mammuthus primigenius
  misc_feature 1..465: note = DNA sequence coding for mammoth myoglobin
  source 1..465: mol_type = other DNA
atgggactcagcgacggggaatgggagttggtgttgaaaacctgggggaaagtggaggctgacatcccgggccatgggctggaagtcttcgtcaggctcttcacaggtcatcccgagaccctggagaagttcgacaagtttaagcacctgaagacagagggcgagatgaaggcctccgaggacctgaagaagcaaggtgttactgtgctcactgccctggggggcatcctcaagaagaaagggcatcaccaggcggagattcagcccctggcccagtctcatgccaccaagcacaagatccccatcaagtatctggagttcatctcggacgccatcatccacgttctgcaaagcaagcatcctgcggaatttggcgctgatgcccagggagccatgaaaaaggccttggagctgttccggaatgacattgcggccaagtataaggagctggggttccagggctag

SEQ ID NO: 11 - DNA, 465 bp, Mammuthus trogontherii
  misc_feature 1..465: note = DNA sequence coding for steppe mammoth myoglobin
  source 1..465: mol_type = other DNA
atgggactcagcgacggggaatgggagttggtgttgaaaacctgggggaaagtggaggctgacatcccgggccatgggctggaagtcttcgtcaggctcttcacaggtcatcccgagaccctggagaagttcgacaagtttaagcacctgaagacagagggcgagatgaaggcctccgaggacctgaagaagcaaggtgttactgtgctcactgccctggggggcatcctcaagaagaaagggcatcaccaggcggagattcagcccctggcccattctcatgccaccaagcacaagatccccatcaagtatctggagttcatctcggacgccatcatccacgttctgcaaagcaagcatcctgcggaatttggcgctgatgcccagggagccatgaaaaaggccttggagctgttccggaatgacattgcggccaagtataaggagctggggttccagggctag

SEQ ID NO: 12 - DNA, 465 bp, Ovis aries
  misc_feature 1..465: note = DNA sequence coding for sheep myoglobin
  source 1..465: mol_type = other DNA
atggggctcagcgacggggaatggcagttggtgctgaatgcctgggggaaggtggaggctgatgtcgcaggccatgggcaggaggtcctcatcaggctcttcacaggtcatcccgagaccctggagaaatttgacaagttcaagcacctgaagacagaggctgagatgaaggcctccgaggacctgaagaagcatggcaacaccgtgctcacggccctagggggtatcctgaaaaagaagggtcaccacgaggcggaggtgaagcacctggccgagtcacacgccaacaagcacaagatccctgtcaagtacctggagttcatctcggacgccatcatccatgttctgcatgccaagcatccttcagacttcggtgctgatgcacagggagccatgagcaaggccctggaactgttccggaacgacatggctgcccagtacaaggtgctgggcttccagggctaa

SEQ ID NO: 13 - DNA, 465 bp, Bos taurus
  misc_feature 1..465: note = DNA sequence coding for cow myoglobin
  source 1..465: mol_type = other DNA
atggggctcagcgacggggaatggcagttggtgctgaatgcctgggggaaggtggaggctgatgtcgcaggccatgggcaggaggtcctcatcaggctcttcacaggtcatcccgagaccctggagaaatttgacaagttcaagcacctgaagacagaggctgagatgaaggcctccgaggacctgaagaagcatggcaacacggtgctcacggccctggggggtatcctgaagaaaaagggtcaccatgaggcagaggtgaagcacctggccgagtcacatgccaacaagcacaagatccctgtcaagtacctggagttcatctcggacgccatcatccatgttctacatgccaagcatccttcagacttcggtgctgatgcccaggctgccatgagcaaggccctggaactgttccggaatgacatggctgcccagtacaaggtgctgggcttccatggctaa

SEQ ID NO: 14 - DNA, 465 bp, Sus scrofa
  misc_feature 1..465: note = DNA sequence coding for pig myoglobin
  source 1..465: mol_type = other DNA
atggggctcagcgacggggaatggcagctggtgctgaacgtctgggggaaggtggaggctgatgtcgcaggccatgggcaggaggtcctcatcaggctctttaagggtcaccccgagaccctggagaaatttgataagtttaagcacctgaagtcagaggatgagatgaaggcctctgaggacctgaagaagcacggcaacacggtgctgactgccctggggggcatccttaagaagaaggggcatcatgaggcagagctgacgcccctggcccaatcgcatgccaccaagcacaagatccctgtcaagtacctggagttcatctcagaagccatcatccaggttctgcagagcaagcatcctggggactttggtgctgacgcccagggagccatgagcaaggccctggaactcttccggaacgacatggcggccaagtacaaggagctgggcttccagggctaa

SEQ ID NO: 15 - DNA, 465 bp, Gallus gallus
  misc_feature 1..465: note = DNA sequence coding for chicken myoglobin
  source 1..465: mol_type = other DNA
atggggctcagcgaccaggagtggcaacaagtcctcaccatctggggaaaagtggaggccgacattgctggccatggacacgaggttctgatgagacttttccatgaccaccctgagactttggatcgctttgataagttcaaaggcctgaagacccctgatcagatgaagggctctgaagatctgaagaaacatggagctactgtcctcacccagcttggcaaaatcctgaagcagaagggtaatcatgagtcagagctgaagcccctggctcaaacccatgccacgaagcacaaaatcccagtcaaatatctggagttcatttctgaagtcattatcaaggtcattgctgaaaaacatgccgcagactttggggccgattcccaggctgccatgaagaaggctctggagttgttccgaaatgacatggccagcaagtacaaggagtttggtttccagggttag

SEQ ID NO: 16 - DNA, 444 bp, Thunnus orientalis
  misc_feature 1..444: note = DNA sequence coding for tuna myoglobin
  source 1..444: mol_type = other DNA
atggctgactttgatgcagttctgaagtgttggggtccagtggaggcggactacaccaccattggaggcctggttctgacccgtttattcaaagagcaccctgagacccagaagctgttccccaaattcgctggcatcgcccaggctgacatagccggtaacgcagctgtttctgctcatggtgccactgtgctgaagaaacttggagagctgctgaaggccaaaggcagtcacgctgccatcctaaaaccactggcaaacagccatgccactaagcacaagattcccattaataacttcaagctgatttctgaggtccttgtgaaggtcatgcatgagaaggcaggactcgatgccggtgggcagacagccctgaggaacgtgatgggtatcatcatcgccgaccttgaggccaactacaaagagctgggcttctctggctga

SEQ ID NO: 17 - protein, 175 aa, Mammuthus primigenius
  REGION 1..175: note = mammoth casein k
MKGFLLVVNILLLPLFLAAEVQNQEESRCLEKDERWFCQKAVKYIPNDYVLKSYYRYEPNYNQFRAAVPINNPYLIYLYPAKQVAVRPHTQIQWQVPSNIYPSPSVPHTYLKPPFIIPPKKTQDKPIIPPTGTVASIEATVEPKVNTVVNAEASSEFIATNTPEATTVPVISPQI

SEQ ID NO: 18 - protein, 260 aa, Mammuthus primigenius
  REGION 1..260: note = mammoth casein beta
MKVFILACLVAFALGRETVENLSSSEIRQFYSEQKPEGVKHEEQQREDEHQNKIQPLFQPQPLVYPFAEPIPYTVFPPNAIPLAQPIVVLPFPQPEVQLPEAKEITFPRQKLMSFLKSPVMPFFDPQPNLGTDLENLHLPLPLLQPLRHQLHQPLAQTPVLPLPLSLPKVLPVPQQVIPYPQRGRPIQNLLYEEPLLDPTRKIYPVAQPLAPVYNPVAYMIGIPCCSTLLTYLHQSSRSQYPIQNKLGYLIAMPKKVRPT

SEQ ID NO: 19 - DNA, 462 bp, synthetic construct
  misc_feature 1..462: note = codon optimized nucleotide sequence encoding for a steppe mammoth myoglobin
  source 1..462: mol_type = other DNA
ggtttgtctgatggtgaatgggagttggttttgaagacttggggtaaagttgaggctgatattcctggtcatggtttggaggtttttgttagattgttcactggtcatccagaaactttggagaagttcgataagttcaaacatttgaagactgagggtgaaatgaaggcttctgaggatttgaaaaagcaaggtgttactgttttgactgctttgggtggtattttgaagaagaaaggtcaccatcaagctgaaattcaaccattggctcactctcatgctactaaacacaagattccaattaagtacttggagttcatttctgatgctattattcacgttttgcaatctaagcatccagctgaatttggtgctgatgctcaaggtgctatgaaaaaggctttggagttgttcagaaacgatattgctgctaaatacaaggagttgggtttccaaggttaa

SEQ ID NO: 20 - DNA, 462 bp, synthetic construct
  misc_feature 1..462: note = codon optimized nucleotide sequence encoding for a sheep myoglobin
  source 1..462: mol_type = other DNA
ggtttgtctgatggtgaatggcaattggttttgaacgcttggggtaaagttgaggctgatgttgctggtcatggtcaagaagttttgattagattgttcactggtcaccctgaaactttggagaagtttgataagttcaaacacttgaagactgaggctgaaatgaaggcttctgaggatttgaaaaagcatggtaacactgttttgactgctttgggtggtattttgaagaagaaaggtcaccatgaagctgaggttaagcacttggctgaatctcacgctaacaagcacaaaattcctgttaagtacttggagttcatttctgatgctattattcatgttttgcacgctaagcatccatctgatttcggtgctgatgctcaaggtgctatgtctaaggctttggaattgttcagaaacgatatggctgctcaatacaaggttttgggtttccaaggttaa

SEQ ID NO: 21 - DNA, 462 bp, synthetic construct
  misc_feature 1..462: note = codon optimized nucleotide sequence encoding for a cattle myoglobin
  source 1..462: mol_type = other DNA
ggtttgtctgatggtgaatggcaattggttttgaacgcttggggtaaagttgaggctgatgttgctggtcatggtcaagaggttttgattagattgttcactggtcatccagaaactttggagaagtttgataaattcaagcacttgaagactgaagctgagatgaaggcttctgaggatttgaaaaagcacggtaacactgttttgactgctttgggtggtattttgaagaaaaagggtcaccatgaggctgaagttaagcacttggctgaatctcatgctaacaagcacaaaattcctgttaagtacttggagttcatttctgatgctattattcacgttttgcatgctaagcacccatctgatttcggtgctgatgctcaagctgctatgtctaaggctttggagttgtttagaaacgatatggctgctcaatacaaggttttgggtttccacggttaa

SEQ ID NO: 22 - DNA, 462 bp, synthetic construct
  misc_feature 1..462: note = codon optimized nucleotide sequence encoding for a pig myoglobin
  source 1..462: mol_type = other DNA
ggtttgtctgatggtgaatggcaattggttttgaacgtttggggtaaagttgaggctgatgttgctggtcatggtcaagaggttttgattagattgttcaagggtcatccagaaactttggagaaatttgataagttcaagcacttgaagtctgaagatgagatgaaggcttctgaggatttgaagaaacacggtaacactgttttgactgctttgggtggtattttgaaaaagaaaggtcaccatgaagctgagttgactccattggctcaatctcatgctactaagcacaagattccagttaaatacttggagtttatttctgaggctattattcaagttttgcaatctaagcatcctggtgacttcggtgctgatgctcaaggtgctatgtctaaggctttggagttgttcagaaacgatatggctgctaagtacaaggagttgggtttccaaggttaa

SEQ ID NO: 23 - DNA, 462 bp, synthetic construct
  misc_feature 1..462: note = codon optimized nucleotide sequence encoding for a chicken myoglobin
  source 1..462: mol_type = other DNA
ggtttgtctgatcaagaatggcaacaagttttgactatttggggtaaagttgaggctgatattgctggtcatggtcacgaggttttgatgagattgttccatgatcacccagaaactttggatagattcgataagttcaagggtttgaaaactccagatcaaatgaagggttctgaggatttgaagaaacacggtgctactgttttgactcaattgggtaaaattttgaagcaaaaaggtaaccatgagtctgaattgaagccattggctcaaactcacgctactaagcacaagattcctgttaagtacttggagttcatttctgaggttattattaaggttattgctgaaaagcatgctgctgatttcggtgctgattctcaagctgctatgaaaaaggctttggaattgttcagaaacgatatggcttctaaatacaaggagttcggttttcaaggttaa

SEQ ID NO: 24 - DNA, 441 bp, synthetic construct
  misc_feature 1..441: note = codon optimized nucleotide sequence encoding for a tuna myoglobin
  source 1..441: mol_type = other DNA
gctgatttcgatgctgttttgaagtgttggggtccagttgaagctgattacactactattggtggtttggttttgactagattgttcaaggagcatccagaaactcaaaagttgtttccaaagttcgctggtattgctcaagctgatattgctggtaacgctgctgtttctgctcatggtgctactgttttgaagaaattgggtgaattgttgaaggctaaaggttctcatgctgctattttgaagccattggctaactctcacgctactaaacacaagattccaattaacaatttcaagttgatttctgaggttttggttaaggttatgcacgaaaaggctggtttggatgctggtggtcaaactgctttgagaaacgttatgggtattattattgctgatttggaagctaactacaaggaattgggtttttctggttaa

SEQ ID NO: 25 - DNA, 729 bp, synthetic construct
  misc_feature 1..729: note = gene construct for expressing a steppe mammoth myoglobin
  source 1..729: mol_type = other DNA
atgagattcccatctattttcactgctgttttgttcgctgcttcttctgctttggctgctccagttaatactactactgaggatgaaactgctcaaattccagctgaagctgttattggttactctgatttggagggtgacttcgatgttgctgttttgccattctctaactctactaataacggtttgttgtttattaacactactattgcttctattgctgctaaggaagagggtgtttctttggagaagagagaagctgaagctggtttgtctgatggtgaatgggagttggttttgaagacttggggtaaagttgaggctgatattcctggtcatggtttggaggtttttgttagattgttcactggtcatccagaaactttggagaagttcgataagttcaaacatttgaagactgagggtgaaatgaaggcttctgaggatttgaaaaagcaaggtgttactgttttgactgctttgggtggtattttgaagaagaaaggtcaccatcaagctgaaattcaaccattggctcactctcatgctactaaacacaagattccaattaagtacttggagttcatttctgatgctattattcacgttttgcaatctaagcatccagctgaatttggtgctgatgctcaaggtgctatgaaaaaggctttggagttgttcagaaacgatattgctgctaaatacaaggagttgggtttccaaggttaa

SEQ ID NO: 26 - DNA, 729 bp, synthetic construct
  misc_feature 1..729: note = gene construct for expressing a sheep myoglobin
  source 1..729: mol_type = other DNA
atgagattcccatctattttcactgctgttttgttcgctgcttcttctgctttggctgctcctgttaatactactactgaggatgaaactgctcaaattcctgctgaagctgttattggttattctgatttggagggtgacttcgatgttgctgttttgcctttctctaactctactaataacggtttgttgttcattaacactactattgcttctattgctgctaaggaagagggtgtttctttggaaaagagagaggctgaagctggtttgtctgatggtgaatggcaattggttttgaacgcttggggtaaagttgaggctgatgttgctggtcatggtcaagaagttttgattagattgttcactggtcaccctgaaactttggagaagtttgataagttcaaacacttgaagactgaggctgaaatgaaggcttctgaggatttgaaaaagcatggtaacactgttttgactgctttgggtggtattttgaagaagaaaggtcaccatgaagctgaggttaagcacttggctgaatctcacgctaacaagcacaaaattcctgttaagtacttggagttcatttctgatgctattattcatgttttgcacgctaagcatccatctgatttcggtgctgatgctcaaggtgctatgtctaaggctttggaattgttcagaaacgatatggctgctcaatacaaggttttgggtttccaaggttaa

SEQ ID NO: 27 - DNA, 729 bp, synthetic construct
  misc_feature 1..729: note = gene construct for expressing a cattle myoglobin
  source 1..729: mol_type = other DNA
atgagattcccttctattttcactgctgttttgttcgctgcttcttctgctttggctgctccagttaacactactactgaggatgaaactgctcaaattccagctgaagctgttattggttactctgatttggagggtgacttcgatgttgctgttttgccattctctaactctactaacaatggtttgttgttcattaacactactattgcttctattgctgctaaggaggaaggtgtttctttggagaagagagaagctgaggctggtttgtctgatggtgaatggcaattggttttgaacgcttggggtaaagttgaggctgatgttgctggtcatggtcaagaggttttgattagattgttcactggtcatccagaaactttggagaagtttgataaattcaagcacttgaagactgaagctgagatgaaggcttctgaggatttgaaaaagcacggtaacactgttttgactgctttgggtggtattttgaagaaaaagggtcaccatgaggctgaagttaagcacttggctgaatctcatgctaacaagcacaaaattcctgttaagtacttggagttcatttctgatgctattattcacgttttgcatgctaagcacccatctgatttcggtgctgatgctcaagctgctatgtctaaggctttggagttgtttagaaacgatatggctgctcaatacaaggttttgggtttccacggttaa

SEQ ID NO: 28 - DNA, 729 bp, synthetic construct
  misc_feature 1..729: note = gene construct for expressing a pig myoglobin
  source 1..729: mol_type = other DNA
atgagattcccatctattttcactgctgttttgttcgctgcttcttctgctttggctgctccagttaacactactactgaggatgaaactgctcaaattccagctgaagctgttattggttactctgatttggagggtgacttcgatgttgctgttttgccattctctaattctactaacaatggtttgttgttcattaacactactattgcttctattgctgctaaggaagagggtgtttctttggagaagagagaagctgaggctggtttgtctgatggtgaatggcaattggttttgaacgtttggggtaaagttgaggctgatgttgctggtcatggtcaagaggttttgattagattgttcaagggtcatccagaaactttggagaaatttgataagttcaagcacttgaagtctgaagatgagatgaaggcttctgaggatttgaagaaacacggtaacactgttttgactgctttgggtggtattttgaaaaagaaaggtcaccatgaagctgagttgactccattggctcaatctcatgctactaagcacaagattccagttaaatacttggagtttatttctgaggctattattcaagttttgcaatctaagcatcctggtgacttcggtgctgatgctcaaggtgctatgtctaaggctttggagttgttcagaaacgatatggctgctaagtacaaggagttgggtttccaaggttaa

SEQ ID NO: 29 - DNA, 729 bp, synthetic construct
  misc_feature 1..729: note = gene construct for expressing a chicken myoglobin
  source 1..729: mol_type = other DNA
atgagattcccatctattttcactgctgttttgttcgctgcttcttctgctttggctgctccagttaacactactactgaagatgagactgctcaaattcctgctgaagctgttattggttactctgatttggagggtgacttcgatgttgctgttttgcctttttctaactctactaacaatggtttgttgttcattaacactactattgcttctattgctgctaaggaagagggtgtttctttggagaaaagagaggctgaagctggtttgtctgatcaagaatggcaacaagttttgactatttggggtaaagttgaggctgatattgctggtcatggtcacgaggttttgatgagattgttccatgatcacccagaaactttggatagattcgataagttcaagggtttgaaaactccagatcaaatgaagggttctgaggatttgaagaaacacggtgctactgttttgactcaattgggtaaaattttgaagcaaaaaggtaaccatgagtctgaattgaagccattggctcaaactcacgctactaagcacaagattcctgttaagtacttggagttcatttctgaggttattattaaggttattgctgaaaagcatgctgctgatttcggtgctgattctcaagctgctatgaaaaaggctttggaattgttcagaaacgatatggcttctaaatacaaggagttcggttttcaaggttaa

SEQ ID NO: 30 - DNA, 708 bp, synthetic construct
  misc_feature 1..708: note = gene construct for expressing a tuna myoglobin
  source 1..708: mol_type = other DNA
atgagattcccttctattttcactgctgttttgtttgctgcttcttctgctttggctgctccagttaacactactactgaagatgagactgctcaaattccagctgaagctgttattggttactctgatttggagggtgacttcgatgttgctgttttgccattctctaactctactaataacggtttgttgtttattaacactactattgcttctattgctgctaaggaggaaggtgtttctttggagaaaagagaagctgaggctgctgatttcgatgctgttttgaagtgttggggtccagttgaagctgattacactactattggtggtttggttttgactagattgttcaaggagcatccagaaactcaaaagttgtttccaaagttcgctggtattgctcaagctgatattgctggtaacgctgctgtttctgctcatggtgctactgttttgaagaaattgggtgaattgttgaaggctaaaggttctcatgctgctattttgaagccattggctaactctcacgctactaaacacaagattccaattaacaatttcaagttgatttctgaggttttggttaaggttatgcacgaaaaggctggtttggatgctggtggtcaaactgctttgagaaacgttatgggtattattattgctgatttggaagctaactacaaggaattgggtttttctggttaa

SEQ ID NO: 31 - protein, 13 aa, synthetic construct
  REGION 1..13: note = peptide in MS analysis
MGLSDGEWELVLK

SEQ ID NO: 32 - protein, 12 aa, synthetic construct
  REGION 1..12: note = peptide in MS analysis
GLSDGEWELVLK

SEQ ID NO: 33 - protein, 11 aa, synthetic construct
  REGION 1..11: note = peptide in MS analysis
LSDGEWELVLK

SEQ ID NO: 34 - protein, 20 aa, synthetic construct
  REGION 1..20: note = peptide in MS analysis
KTWGKVEADIPGHGLEVFVR

SEQ ID NO: 35 - protein, 14 aa, synthetic construct
  REGION 1..14: note = peptide in MS analysis
KVEADIPGHGLEVF

SEQ ID NO: 36 - protein, 16 aa, synthetic construct
  REGION 1..16: note = peptide in MS analysis
KVEADIPGHGLEVFVR

SEQ ID NO: 37 - protein, 13 aa, synthetic construct
  REGION 1..13: note = peptide in MS analysis
ADIPGHGLEVFVR

SEQ ID NO: 38 - protein, 12 aa, synthetic construct
  REGION 1..12: note = peptide in MS analysis
DIPGHGLEVFVR

SEQ ID NO: 39 - protein, 11 aa, synthetic construct
  REGION 1..11: note = peptide in MS analysis
RLFTGHPETLE

SEQ ID NO: 40 - protein, 12 aa, synthetic construct
  REGION 1..12: note = peptide in MS analysis
RLFTGHPETLEK

SEQ ID NO: 41 - protein, 14 aa, synthetic construct
  REGION 1..14: note = peptide in MS analysis
RLFTGHPETLEKFD

SEQ ID NO: 42 - protein, 15 aa, synthetic construct
  REGION 1..15: note = peptide in MS analysis
RLFTGHPETLEKFDK

SEQ ID NO: 43 - protein, 17 aa, synthetic construct
  REGION 1..17: note = peptide in MS analysis
RLFTGHPETLEKFDKFK

SEQ ID NO: 44 - protein, 11 aa, synthetic construct
  REGION 1..11: note = peptide in MS analysis
LFTGHPETLEK

SEQ ID NO: 45 - protein, 14 aa, synthetic construct
  REGION 1..14: note = peptide in MS analysis
LFTGHPETLEKFDK

SEQ ID NO: 46 - protein, 12 aa, synthetic construct
  REGION 1..12: note = peptide in MS analysis
TGHPETLEKFDK

SEQ ID NO: 47 - protein, 10 aa, synthetic construct
  REGION 1..10: note = peptide in MS analysis
KHLKTEGEMK

SEQ ID NO: 48 - protein, 14 aa, synthetic construct
  REGION 1..14: note = peptide in MS analysis
KTEGEMKASEDLKK

SEQ ID NO: 49 - protein, 11 aa, synthetic construct
  REGION 1..11: note = peptide in MS analysis
KKQGVTVLTAL

SEQ ID NO: 50 - protein, 16 aa, synthetic construct
  REGION 1..16: note = peptide in MS analysis
KKQGVTVLTALGGILK

SEQ ID NO: 51 - protein, 10 aa, synthetic construct
  REGION 1..10: note = peptide in MS analysis
KQGVTVLTAL

SEQ ID NO: 52 - protein, 15 aa, synthetic construct
  REGION 1..15: note = peptide in MS analysis
KQGVTVLTALGGILK

SEQ ID NO: 53 - protein, 16 aa, synthetic construct
  REGION 1..16: note = peptide in MS analysis
KQGVTVLTALGGILKK

SEQ ID NO: 54 - protein, 14 aa, synthetic construct
  REGION 1..14: note = peptide in MS analysis
QGVTVLTALGGILK

SEQ ID NO: 55 - protein, 13 aa, synthetic construct
  REGION 1..13: note = peptide in MS analysis
GVTVLTALGGILK

SEQ ID NO: 56 - protein, 10 aa, synthetic construct
  REGION 1..10: note = peptide in MS analysis
VLTALGGILK

SEQ ID NO: 57 - protein, 10 aa, synthetic construct
  REGION 1..10: note = peptide in MS analysis
LTALGGILKK

SEQ ID NO: 58 - protein, 9 aa, synthetic construct
  REGION 1..9: note = peptide in MS analysis
TALGGILKK

SEQ ID NO: 59 - protein, 13 aa, synthetic construct
  REGION 1..13: note = peptide in MS analysis
KKKGHHQAEIQPL

SEQ ID NO: 60 - protein, 15 aa, synthetic construct
  REGION 1..15: note = peptide in MS analysis
KKKGHHQAEIQPLAH

SEQ ID NO: 61 - protein, 20 aa, synthetic construct
  REGION 1..20: note = peptide in MS analysis
KKKGHHQAEIQPLAHSHATK

SEQ ID NO: 62 - protein, 12 aa, synthetic construct
  REGION 1..12: note = peptide in MS analysis
KKGHHQAEIQPL

SEQ ID NO: 63 - protein, 14 aa, synthetic construct
  REGION 1..14: note = peptide in MS analysis
KKGHHQAEIQPLAH

SEQ ID NO: 64 - protein, 19 aa, synthetic construct
  REGION 1..19: note = peptide in MS analysis
KKGHHQAEIQPLAHSHATK

SEQ ID NO: 65 - protein, 11 aa, synthetic construct
  REGION 1..11: note = peptide in MS analysis
KGHHQAEIQPL

SEQ ID NO: 66 - protein, 13 aa, synthetic construct
  REGION 1..13: note = peptide in MS analysis
KGHHQAEIQPLAH

SEQ ID NO: 67 - protein, 18 aa, synthetic construct
  REGION 1..18: note = peptide in MS analysis
KGHHQAEIQPLAHSHATK

SEQ ID NO: 68 - protein, 16 aa, synthetic construct
  REGION 1..16: note = peptide in MS analysis
HHQAEIQPLAHSHATK

SEQ ID NO: 69 - protein, 15 aa, synthetic construct
  REGION 1..15: note = peptide in MS analysis
HQAEIQPLAHSHATK

SEQ ID NO: 70 - protein, 13 aa, synthetic construct
  REGION 1..13: note = peptide in MS analysis
AEIQPLAHSHATK

SEQ ID NO: 71 - protein, 12 aa, synthetic construct
  REGION 1..12: note = peptide in MS analysis
KYLEFISDAIIH

SEQ ID NO: 72 - protein, 17 aa, synthetic construct
  REGION 1..17: note = peptide in MS analysis
KYLEFISDAIIHVLQSK

SEQ ID NO: 73 - protein, 13 aa, synthetic construct
  REGION 1..13: note = peptide in MS analysis
FISDAIIHVLQSK

SEQ ID NO: 74 - protein, 10 aa, synthetic construct
  REGION 1..10: note = peptide in MS analysis
DAIIHVLQSK

SEQ ID NO: 75 - protein, 11 aa, synthetic construct
  REGION 1..11: note = peptide in MS analysis
KHPAEFGADAQ

SEQ ID NO: 76 - protein, 15 aa, synthetic construct
  REGION 1..15: note = peptide in MS analysis
KHPAEFGADAQGAMK

SEQ ID NO: 77 - protein, 16 aa, synthetic construct
  REGION 1..16: note = peptide in MS analysis
KHPAEFGADAQGAMKK

SEQ ID NO: 78 - protein, 13 aa, synthetic construct
  REGION 1..13: note = peptide in MS analysis
PAEFGADAQGAMK

SEQ ID NO: 79 - protein, 14 aa, synthetic construct
  REGION 1..14: note = peptide in MS analysis
PAEFGADAQGAMKK

SEQ ID NO: 80 - protein, 13 aa, synthetic construct
  REGION 1..13: note = peptide in MS analysis
KALELFRNDIAAK